European Patent Application EP 4 556 485 A1, published May 21, 2025. Title: NOVEL POLYPEPTIDE HAVING GLUCANASE ACTIVITY. Applicant: 씨제이제일제당 주식회사. The sequence listing filed with the application follows.

SEQUENCE LISTING (4 sequences)

SEQ ID NO: 1 - DNA, 648 bp, synthetic construct
  source 1..648: mol_type = other DNA
gggactgcgtggaacgggagccatgatgtgatggacttcaattatcatgagagtaatagattcgagatgagcaactggccaaatggagaaatgtttaactgtagatggactcccaacaacgttaaattcgaaaatggcaagctgaagctgaccatagaccgggacggttcgggctacacctgtggtgagtaccgtacaaagaactattatggctatgggatgttccaggtaaatatgaaacccatcaaaaatcccggcgtcgtgtcttcgttctttacctacactggtccaagcgatggaacaaaatgggatgagattgatattgagttcctgggatatgatacaactaaggtccaattcaactattatacaaatggtcaaggccatcacgagcacattcattatttggggttcgacgcttctcaaggatttcacacatacgggtttttttgggctcgtaattcgataacttggtacgtcgatgggactgcagtttatacagcttatgataacatacccgatacaccggggaagatcatgatgaatgcatggaatggaataggggtcgatgattggctgcgtcctttcaacggccgcacgaacatttccgcgtattatgattgggtatcctatgacgctccccgcaac

SEQ ID NO: 2 - protein, 216 aa, synthetic construct
GTAWNGSHDVMDFNYHESNRFEMSNWPNGEMFNCRWTPNNVKFENGKLKLTIDRDGSGYTCGEYRTKNYYGYGMFQVNMKPIKNPGVVSSFFTYTGPSDGTKWDEIDIEFLGYDTTKVQFNYYTNGQGHHEHIHYLGFDASQGFHTYGFFWARNSITWYVDGTAVYTAYDNIPDTPGKIMMNAWNGIGVDDWLRPFNGRTNISAYYDWVSYDAPRN

SEQ ID NO: 3 - DNA, 645 bp, synthetic construct
  source 1..645: mol_type = other DNA
gctactgcggttaatacaccctttgtcgctgattttaactatcatgatagctctcagtgggaaatgtccaattggccgaacggcgagatgttcaactgccgttggaccccgaataacgttaaattcgagaacggcaagctcaagttgaccattgacagagatggcagcggttacacctgtggtgagtatcgtactaagaactatttcggctacggctactacgaggttcgtatgaaaccgattaaaaatccaggtgtagtgagctcgttcttcacgtacacgggtccgtctgatggcaccaaatgggacgaaatcgacatcgaatttctgggttatgataccaccaaggttcagtttaattattataccaacggtcagggtggtcatgaacatattcattatctgggttttgacgcaagccaagatttccacacctacggcttcttttgggcgcgtaacagcatcacctggtatgtggacggcaccgcggtgtataccgcgactgataacattccggataccccgggtaagatcatgatgaacgcgtggaacggaatcggtgtggatgactggctgcgcccttttaacggccgtaccaatattagcgcgtattacgagtacgttaagtattacccgaatggcaac

SEQ ID NO: 4 - protein, 215 aa, synthetic construct
ATAVNTPFVADFNYHDSSQWEMSNWPNGEMFNCRWTPNNVKFENGKLKLTIDRDGSGYTCGEYRTKNYFGYGYYEVRMKPIKNPGVVSSFFTYTGPSDGTKWDEIDIEFLGYDTTKVQFNYYTNGQGGHEHIHYLGFDASQDFHTYGFFWARNSITWYVDGTAVYTATDNIPDTPGKIMMNAWNGIGVDDWLRPFNGRTNISAYYEYVKYYPNGN